European Patent Application EP 4 268 832 A2, published November 1, 2023. Title: NUCLEIC ACID MOLECULES FOR PSEUDOURIDYLATION. Applicant: ProQR Therapeutics II B.V. Application EP. The sequence listing filed with the application follows.

SEQUENCE LISTING (42 sequences)

SEQ ID NO: 1 - RNA, 30 nt, synthetic construct
  misc_feature 1..30: note = "Description of Artificial Sequence: Synthetic oligonucleotide"
  misc_feature 1..30: note = "RNA target substrate"
  source 1..30: mol_type = other RNA
aggggaaccccacagtcgaaccaaaacaaa

SEQ ID NO: 2 - RNA, 30 nt, synthetic construct
  misc_feature 1..30: note = "Description of Artificial Sequence: Synthetic oligonucleotide"
  misc_feature 1..30: note = "RNA target substrate"
  source 1..30: mol_type = other RNA
gacaatatagttctttgagaaggtggaatc

SEQ ID NO: 3 - RNA, 30 nt, synthetic construct
  misc_feature 1..30: note = "Description of Artificial Sequence: Synthetic oligonucleotide"
  misc_feature 1..30: note = "RNA target substrate"
  source 1..30: mol_type = other RNA
gatggagaacaactctaggcagaggtctca

SEQ ID NO: 4 - RNA, 61 nt, Homo sapiens
  source 1..61: mol_type = other RNA
gggtccgccttgagtgcccgggtgagaagcatgatcccgggtaattatggcggacccacag

SEQ ID NO: 5 - RNA, 128 nt, Homo sapiens
  source 1..128: mol_type = other RNA
gtgcacatttcattgacctgctttcttttatgtgagtagtgttatttcttatgtgctatacaaataattgaaggctaattagcagtataactataaatagtaatgctgcctgtgtccttcagacaaaa

SEQ ID NO: 6 - RNA, 28 nt, synthetic construct
  misc_feature 1..28: note = "Description of Artificial Sequence: Synthetic oligonucleotide"
  misc_feature 1..28: note = "Substrate RNA"
  source 1..28: mol_type = other RNA
  modified_base 14: mod_base = p
  rRNA 1..28: note = rRNA
aaagtgaagaaatncaatgaagcgcggg

SEQ ID NO: 7 - RNA, 24 nt, synthetic construct
  misc_feature 1..24: note = "Description of Artificial Sequence: Synthetic oligonucleotide"
  misc_feature 1..24: note = "Substrate RNA"
  source 1..24: mol_type = other RNA
  modified_base 12: mod_base = p
  rRNA 1..24: note = rRNA
gaatccgactgnttaattaaaaca

SEQ ID NO: 8 - RNA, 65 nt, synthetic construct
  misc_feature 1..65: note = "Description of Artificial Sequence: Synthetic oligonucleotide"
  misc_feature 1..65: note = "psEON"
  source 1..65: mol_type = other RNA
ggaattgaaggctggttcgcagtataactataaatagtaatgctgcctgtgtccttcagacaaaa

SEQ ID NO: 9 - RNA, 65 nt, synthetic construct
  misc_feature 1..65: note = "Description of Artificial Sequence: Synthetic oligonucleotide"
  misc_feature 1..65: note = "psEON"
  source 1..65: mol_type = other RNA
ggaattgaaggcccttctgcagtataactataaatagtaatgctgcaagaacccttcagacaaaa

SEQ ID NO: 10 - RNA, 66 nt, synthetic construct
  misc_feature 1..66: note = "Description of Artificial Sequence: Synthetic oligonucleotide"
  misc_feature 1..66: note = "psEON"
  source 1..66: mol_type = other RNA
ggaattgaaggctctgccgcagtataactataaatagtaatgctgcgagttgtccttcagacaaaa

SEQ ID NO: 11 - DNA, 5462 bp, synthetic construct
  misc_feature 1..5462: note = "Description of Artificial Sequence: Synthetic polynucleotide"
  misc_feature 1..5462: note = "pugIntron-mIDUA plasmid"
  source 1..5462: mol_type = other DNA
  CDS join(893..985,1150..1371): protein_id = 41; translation = MVHLTPEEKSAVTALWGKVNVDEVGGEALGRLLVVYPWTQRFFESFGDLSTPDAVMGNPKVKAHGKKVLGAFSDGLAHLDNLKGTFATLSELHCDKLHVDPENFR
gcgcccaatacgcaaaccgcctctccccgcgcgttggccgattcattaatgcagctggcacgacaggtttcccgactggaaagcgggcagtgagcgcaacgcaattaatgtgagttagctcactcattaggcaccccacactttatgcttccggctcgtatgttgtgtggaattgtgagcggataacaatttcacacaggaaacagctatgaccatgattacgccaagctcggatcctagagatatactgagtcattagggactttccaatgggttttgcccagtacataaggtcaataggggtgaatcaacaggaaagtcccattggagccaagtacactgagtcaatagggactttccattgggttttgcccagtacaaaaggtcaatagggggtgagtcaatgggtttttcccattattggcacgtacataaggtcaataggggtgagtcattgggtttttccagccaatttaattaaaacgccatgtactttcccaccattgacgtcaatgggctattgaaactaatgcaacgtgacctttaaacggtactttcccatagctgattaatgggaaagtaccgttctcgagccaatacacgtcaatgggaagtgaaagggcagccaaaacgtaacaccgccccggttttcccctggaaattccatattggcacgcattctattggctgagctgcgttctacgtgggtataagaggcgcgaccagcgtcggtaccgtcgcagtcttcggtctgaccaccgtagaacgcagatcgaattgatcccgcgcagacactgaccttcagcgcctcggctccagcgccatggcttccaaggctcgagctcagtacatcaagagcttcgtggagcgcgtgctgaagaacgagcagtacatggtgcacctgactcctgaggagaagtctgccgttactgccctgtggggcaaggtgaacgtggatgaagttggtggtgaggccctgggcaggtaagtcgacgtgggagattctgcctcggacagagagaaactctgctgtgtctgagagttgatctccctatagtgaccctgccttcttgccccgggacgaaatgagagaaatcgtaacgggagtttacgaggcagacaggttgactctctcttttcccctgcaggctgctggtggtctacccttggacccagaggttctttgagtcctttggggatctgtccactcctgatgctgttatgggcaaccctaaggtgaaggctcatggcaagaaagtgctcggtgcctttagtgatggcctggctcacctggacaacctcaagggcacctttgccacactgagtgagctgcactgtgacaagctgcacgtggatcctgagaacttcagggtgagtctgatgggcacctcctgggtttccttcccctggctattctgctcaaccttcctatcagaaaaaaaggggaagcgattctagggagcagtctccatgactgtgtgtggagtgttgacaagagttcggatattttattctctactcagaattgctgctccccctcactctgttctgtgttgtcatttcctctttctttggtaagcttttaatttccagttgcattttactaaattaattaagctggttatttacttcccatcctgatatcagcttcccctcctcctttcctcccagtccttctctctctcctctctctttctctaatcctttcctttccctcagttcatttcttcttctttgatctacgtttgtttgtctttttaaatattgccttgtaacttgctcagaggacaaggaagatatgtccctgtttcttctcatagctctcaagaatagtagcataattggcttttatgccagggtgacaggggaagaatatattttacatataaattctgtttgacataggattcttataataatttgtcagtagtttaaggttgcaaacaaatgtctttgtaaataagcctgcagtatctggtatttttgctctacagttatgttgatggttcttccatattcccacagctcctgggcaatatgatcgtgattgtgctgggccaccacctgggcaaggatttcacccccgctgcacaggctgccttccagaaggtggtggctggagtggccactgccctggctcacaagtaccactaaaccccctttcctgctcttgcctgtgaacaatggttaattgttcccaagagagcatctgtcagttgttggcaaaatgatagacatttgaaaatctgtcttctgacaaataaaaagcatttatgttcactgcaatgatgttttaaattatttgtctgtgtcatagaagggtttatgctaagttttcaagatacaaagaagtgagggttcaggtctgaccttggggaaataaatgaattacacttcaaatgtgtgggacagcaagcagtaagccacagatcctattgccatgccctaaacactcagagaaaaattcaacaaatggtttcatttacacactacattatgattacattttatgtaaattatttgtttttttctactcttccacataaatgtctttttttcctcttacctacccagcacttcacagttctcaagccaataatttttcttttgtaaaactaccattattctctaaacttttccctctgtgtttaccaagcaacattatttatcttttcataaatcctgttgccttagacagcttcagtagcaatagaggtaggattaaggagagaatagaagtgccctgtttgtcataccatgcctgcacagtcaatagtcactatgggatttcaaatggcactttgcctgggacctttacacttcacaccatactctggcttgagttaggagttaagaatgagagaaatataagtctagagagaataagaatatctagtttttaaggctcattactggggtcttatgaaatttccataataccctgtaaatggaagcatttattttttcaataaatctatcttgaatatccagtgtgggttaggattaaatctctccttcatacagttggactgcttttatttatatggagttactagagttaattcactggccgtcgttttacaacgtcgtgactgggaaaaccctggcgttacccaacttaatcgccttgcagcacatccccctttcgccagctggcgtaatagcgaagaggcccgcaccgatcgcccttcccaacagttgcgcagcctgaatggcgaatggcgcctgatgcggtattttctccttacgcatctgtgcggtatttcacaccgcatatggtgcactctcagtacaatctgctctgatgccgcatagttaagccagccccgacacccgccaacacccgctgacgcgccctgacgggcttgtctgctcccggcatccgcttacagacaagctgtgaccgtctccgggagctgcatgtgtcagaggttttcaccgtcatcaccgaaacgcgcgagacgaaagggcctcgtgatacgcctatttttataggttaatgtcatgataataatggtttcttagacgtcaggtggcacttttcggggaaatgtgcgcggaacccctatttgtttatttttctaaatacattcaaatatgtatccgctcatgagacaataaccctgataaatgcttcaataatattgaaaaaggaagagtatgagtattcaacatttccgtgtcgcccttattcccttttttgcggcattttgccttcctgtttttgctcacccagaaacgctggtgaaagtaaaagatgctgaagatcagttgggtgcacgagtgggttacatcgaactggatctcaacagcggtaagatccttgagagttttcgccccgaagaacgttttccaatgatgagcacttttaaagttctgctatgtggcgcggtattatcccgtattgacgccgggcaagagcaactcggtcgccgcatacactattctcagaatgacttggttgagtactcaccagtcacagaaaagcatcttacggatggcatgacagtaagagaattatgcagtgctgccataaccatgagtgataacactgcggccaacttacttctgacaacgatcggaggaccgaaggagctaaccgcttttttgcacaacatgggggatcatgtaactcgccttgatcgttgggaaccggagctgaatgaagccataccaaacgacgagcgtgacaccacgatgcctgtagcaatggcaacaacgttgcgcaaactattaactggcgaactacttactctagcttcccggcaacaattaatagactggatggaggcggataaagttgcaggaccacttctgcgctcggcccttccggctggctggtttattgctgataaatctggagccggtgagcgtgggtctcgcggtatcattgcagcactggggccagatggtaagccctcccgtatcgtagttatctacacgacggggagtcaggcaactatggatgaacgaaatagacagatcgctgagataggtgcctcactgattaagcattggtaactgtcagaccaagtttactcatatatactttagattgatttaaaacttcatttttaatttaaaaggatctaggtgaagatcctttttgataatctcatgaccaaaatcccttaacgtgagttttcgttccactgagcgtcagaccccgtagaaaagatcaaaggatcttcttgagatcctttttttctgcgcgtaatctgctgcttgcaaacaaaaaaaccaccgctaccagcggtggtttgtttgccggatcaagagctaccaactctttttccgaaggtaactggcttcagcagagcgcagataccaaatactgtccttctagtgtagccgtagttaggccaccacttcaagaactctgtagcaccgcctacatacctcgctctgctaatcctgttaccagtggctgctgccagtggcgataagtcgtgtcttaccgggttggactcaagacgatagttaccggataaggcgcagcggtcgggctgaacggggggttcgtgcacacagcccagcttggagcgaacgacctacaccgaactgagatacctacagcgtgagctatgagaaagcgccacgcttcccgaagggagaaaggcggacaggtatccggtaagcggcagggtcggaacaggagagcgcacgagggagcttccagggggaaacgcctggtatctttatagtcctgtcgggtttcgccacctctgacttgagcgtcgatttttgtgatgctcgtcaggggggcggagcctatggaaaaacgccagcaacgcggcctttttacggttcctggccttttgctggccttttgctcacatgttctttcctgcgttatcccctgattctgtggataaccgtattaccgcctttgagtgagctgataccgctcgccgcagccgaacgaccgagcgcagcgagtcagtgagcgaggaagcggaaga

SEQ ID NO: 12 - DNA, 4974 bp, synthetic construct
  misc_feature 1..4974: note = "Description of Artificial Sequence: Synthetic polynucleotide"
  misc_feature 1..4974: note = "pFLAG-Globin39ter plasmid"
  source 1..4974: mol_type = other DNA
ccattcgccattcaggctgcgcaactgttgggaagggcgatcggtgcgggcctcttcgctattacgccagctggcgaaagggggatgtgctgcaaggcgattaagttgggtaacgccagggttttcccagtcacgacgttgtaaaacgacggccagtgccaagctgatctatacattgaatcaatattggcaattagccatattagtcattggttatatagcataaatcaatattggctattggccattgcatacgttgtatctatatcataatatgtacatttatattggctcatgtccaatatgaccgccatgttgacattgattattgactagttattaatagtaatcaattacggggtcattagttcatagcccatatatggagttccgcgttacataacttacggtaaatggcccgcctggctgaccgcccaacgacccccgcccattgacgtcaataatgacgtatgttcccatagtaacgccaatagggactttccattgacgtcaatgggtggagtatttacggtaaactgcccacttggcagtacatcaagtgtatcatatgccaagtccgccccctattgacgtcaatgacggtaaatggcccgcctggcattatgcccagtacatgaccttacgggactttcctacttggcagtacatctacgtattagtcatcgctattaccatggtgatgcggttttggcagtacaccaatgggcgtggatagcggtttgactcacggggatttccaagtctccaccccattgacgtcaatgggagtttgttttggcaccaaaatcaacgggactttccaaaatgtcgtaataaccccgccccgttgacgcaaatgggcggtaggcgtgtacggtgggaggtctatataagcagagctcgtttagtgaaccgtcagaattgatctaccatggactacaaagacgatgacgacaagcttatggactacaaggacgacgatgacaagcatatggtgcacctgactcctgaggagaagtctgccgttactgccctgtggggcaaggtgaacgtggatgaagttggtggtgaggccctgggcaggttggtatcaaggttacaagacaggtttaaggagaccaatagaaactgggcatgtggagacagagaagactcttgggtttctgataggcactgactctctctgcctattggtctattttcccacccttaggctgctggtggatggagaacaactctaggcagaggtctcaaaatttggggatctgtccactcctgatgctgttatgggcaaccctaaggtgaaggctcatggcaagaaagtgctcggtgcctttagtgatggcctggctcacctggacaacctcaagggcacctttgccacactgagtgagctgcactgtgacaagctgcacgtggatcctgagaacttcagggtgagtctatgggacccttgatgttttctttccccttcttttctatggttaagttcatgtcataggaaggggataagtaacagggtacagtttagaatgggaaacagacgaatgattgcatcagtgtggaagtctcaggatcgttttagtttcttttatttgctgttcataacaattgttttcttttgtttaattcttgctttctttttttttcttctccgcaatttttactattatacttaatgccttaacattgtgtataacaaaaggaaatatctctgagatacattaagtaacttaaaaaaaaactttacacagtctgcctagtacattactatttggaatatatgtgtgcttatttgcatattcataatctccctactttattttcttttatttttaattgatacataatcattatacatatttatgggttaaagtgtaatgttttaatatgtgtacacatattgaccaaatcagggtaattttgcatttgtaattttaaaaaatgctttcttcttttaatatacttttttgtttatcttatttctaatactttccctaatctctttctttcagggcaataatgatacaatgtatcatgcctctttgcaccattctaaagaataacagtgataatttctgggttaaggcaatagcaatatctctgcatataaatatttctgcatataaattgtaactgatgtaagaggtttcatattgctaatagcagctacaatccagctaccattctgcttttattttatggttgggataaggctggattattctgagtccaagctaggcccttttgctaatcatgttcatacctcttatcttcctcccacagctcctgggcaacgtgctggtctgtgtgctggcccatcactttggcaaagaattcaccccaccagtgcaggctgcctatcagaaagtggtggctggtgtggctaatgccctggcccacaagtatcactaagctcgctttcttgctgtccaatttctattaaaggttcctttgttccctaagtccaactactaaactgggggatattatgaagggccttgagcatctggattctgcctaataaaaaacatttattttcattgcaatgatgtatttaaattatttctgaatattttactaaaaagggaatgtgggaggtcagtctagaggatcccgggtggcatccctgtgacccctccccagtgcctctcctggccctggaagttgccactccagtgcccaccagccttgtcctaataaaattaagttgcatcattttgtctgactaggtgtccttctataatattatggggtggaggggggtggtatggagcaaggggcaagttgggaagacaacctgtagggcctgcggggtctattgggaaccaagctggagtgcagtggcacaatcttggctcactgcaatctccgcctcctgggttcaagcgattctcctgcctcagcctcccgagttgttgggattccaggcatgcatgaccaggctcagctaatttttgtttttttggtagagacggggtttcaccatattggccaggctggtctccaactcctaatctcaggtgatctacccaccttggcctcccaaattgctgggattacaggcgtgaaccactgctcccttccctgtccttctgattttaaaataactataccagcaggaggacgtccagacacagcataggctacctggccatgcccaaccggtgggacatttgagttgcttgcttggcactgtcctctcatgcgttgggtccactcagtagatgcctgttgaattgggtacgcggccagcttggctgtggaatgtgtgtcagttagggtgtggaaagtccccaggctccccagcaggcagaagtatgcaaagcatgcatctcaattagtcagcaaccaggtgtggaaagtccccaggctccccagcaggcagaagtatgcaaagcatgcatctcaattagtcagcaaccatagtcccgcccctaactccgcccatcccgcccctaactccgcccagttccgcccattctccgccccatggctgactaattttttttatttatgcagaggccgaggccgcctcggcctctgagctattccagaagtagtgaggaggcttttttggaggcctaggcttttgcaaaaagctcctcgaggaactgaaaaaccagaaagttaattccctatagtgagtcgtattaaattcgtaatcatgtcatagctgtttcctgtgtgaaattgttatccgctcacaattccacacaacatacgagccggaagcataaagtgtaaagcctggggtgcctaatgagtgagctaactcacattaattgcgttgcgctcactgcccgctttccagtcgggaaacctgtcgtgccagctgcattaatgaatcggccaacgcgcggggagaggcggtttgcgtattgggcgctcttccgcttcctcgctcactgactcgctgcgctcggtcgttcggctgcggcgagcggtatcagctcactcaaaggcggtaatacggttatccacagaatcaggggataacgcaggaaagaacatgtgagcaaaaggccagcaaaaggccaggaaccgtaaaaaggccgcgttgctggcgtttttccataggctccgcccccctgacgagcatcacaaaaatcgacgctcaagtcagaggtggcgaaacccgacaggactataaagataccaggcgtttccccctggaagctccctcgtgcgctctcctgttccgaccctgccgcttaccggatacctgtccgcctttctcccttcgggaagcgtggcgctttctcatagctcacgctgtaggtatctcagttcggtgtaggtcgttcgctccaagctgggctgtgtgcacgaaccccccgttcagcccgaccgctgcgccttatccggtaactatcgtcttgagtccaacccggtaagacacgacttatcgccactggcagcagccactggtaacaggattagcagagcgaggtatgtaggcggtgctacagagttcttgaagtggtggcctaactacggctacactagaagaacagtatttggtatctgcgctctgctgaagccagttaccttcggaaaaagagttggtagctcttgatccggcaaacaaaccaccgctggtagcggtggtttttttgtttgcaagcagcagattacgcgcagaaaaaaaggatctcaagaagatcctttgatcttttctacggggtctgacgctcagtggaacgaaaactcacgttaagggattttggtcatgagattatcaaaaaggatcttcacctagatccttttaaattaaaaatgaagttttaaatcaatctaaagtatatatgagtaaacttggtctgacagttaccaatgcttaatcagtgaggcacctatctcagcgatctgtctatttcgttcatccatagttgcctgactccccgtcgtgtagataactacgatacgggagggcttaccatctggccccagtgctgcaatgataccgcgaga

SEQ ID NO: 13 - DNA, 32 bp, synthetic construct
  misc_feature 1..32: note = "Description of Artificial Sequence: Synthetic oligonucleotide"
  misc_feature 1..32: note = "SDM1-GLintron1-Sal-Pst"
  source 1..32: mol_type = other DNA
gtaagtcgacgaattctgcaggctgctggtgg

SEQ ID NO: 14 - DNA, 32 bp, synthetic construct
  misc_feature 1..32: note = "Description of Artificial Sequence: Synthetic oligonucleotide"
  misc_feature 1..32: note = "SDM2-GLintron-Sal-Pst"
  source 1..32: mol_type = other DNA
gcctgcagaattcgtcgacttacctgcccagg

SEQ ID NO: 15 - DNA, 21 bp, synthetic construct
  misc_feature 1..21: note = "Description of Artificial Sequence: Synthetic oligonucleotide"
  misc_feature 1..21: note = "pug-intron-FwdSalI"
  source 1..21: mol_type = other DNA
gttgtcgacgtgggagattct

SEQ ID NO: 16 - DNA, 41 bp, synthetic construct
  misc_feature 1..41: note = "Description of Artificial Sequence: Synthetic oligonucleotide"
  misc_feature 1..41: note = "pug-intron-RevExPstI"
  source 1..41: mol_type = other DNA
aatctgcaggggaaaagagagagtcaacctgtctgcctcgt

SEQ ID NO: 17 - DNA, 58 bp, synthetic construct
  misc_feature 1..58: note = "Description of Artificial Sequence: Synthetic oligonucleotide"
  misc_feature 1..58: note = "SDM-GL39-SWAPto-mmidua-1"
  source 1..58: mol_type = other DNA
tggtggatggagaacaactctaggcagaggtctcaaagtttggggatctgtccactcc

SEQ ID NO: 18 - DNA, 58 bp, synthetic construct
  misc_feature 1..58: note = "Description of Artificial Sequence: Synthetic oligonucleotide"
  misc_feature 1..58: note = "SDM-GL39-SWAPto-mmidua-2"
  source 1..58: mol_type = other DNA
ccaaactttgagacctctgcctagagttgttctccatccaccagcagcctaagggtgg

SEQ ID NO: 19 - DNA, 20 bp, synthetic construct
  misc_feature 1..20: note = "Description of Artificial Sequence: Synthetic oligonucleotide"
  misc_feature 1..20: note = "RLuc-Gl ex1 S4"
  source 1..20: mol_type = other DNA
tctgccgttactgccctgtg

SEQ ID NO: 20 - DNA, 16 bp, synthetic construct
  misc_feature 1..16: note = "Description of Artificial Sequence: Synthetic oligonucleotide"
  misc_feature 1..16: note = "PE-mmiduaPTC+16"
  source 1..16: mol_type = other DNA
ctttgagacctctgcc

SEQ ID NO: 21 - DNA, 41 bp, synthetic construct
  misc_feature 1..41: note = "Description of Artificial Sequence: Synthetic oligonucleotide"
  misc_feature 1..41: note = "pug-intronOPT-RevExPstI"
  source 1..41: mol_type = other DNA
aatctgcaggggaaaagagagagtcagtacctgtctgcctc

SEQ ID NO: 22 - DNA, 5464 bp, synthetic construct
  misc_feature 1..5464: note = "Description of Artificial Sequence: Synthetic polynucleotide"
  misc_feature 1..5464: note = "pugIntronOpt-IDUA"
  source 1..5464: mol_type = other DNA
  CDS join(893..985,1152..1373): protein_id = 42; translation = MVHLTPEEKSAVTALWGKVNVDEVGGEALGRLLVVYPWTQRFFESFGDLSTPDAVMGNPKVKAHGKKVLGAFSDGLAHLDNLKGTFATLSELHCDKLHVDPENFR
gcgcccaatacgcaaaccgcctctccccgcgcgttggccgattcattaatgcagctggcacgacaggtttcccgactggaaagcgggcagtgagcgcaacgcaattaatgtgagttagctcactcattaggcaccccacactttatgcttccggctcgtatgttgtgtggaattgtgagcggataacaatttcacacaggaaacagctatgaccatgattacgccaagctcggatcctagagatatactgagtcattagggactttccaatgggttttgcccagtacataaggtcaataggggtgaatcaacaggaaagtcccattggagccaagtacactgagtcaatagggactttccattgggttttgcccagtacaaaaggtcaatagggggtgagtcaatgggtttttcccattattggcacgtacataaggtcaataggggtgagtcattgggtttttccagccaatttaattaaaacgccatgtactttcccaccattgacgtcaatgggctattgaaactaatgcaacgtgacctttaaacggtactttcccatagctgattaatgggaaagtaccgttctcgagccaatacacgtcaatgggaagtgaaagggcagccaaaacgtaacaccgccccggttttcccctggaaattccatattggcacgcattctattggctgagctgcgttctacgtgggtataagaggcgcgaccagcgtcggtaccgtcgcagtcttcggtctgaccaccgtagaacgcagatcgaattgatcccgcgcagacactgaccttcagcgcctcggctccagcgccatggcttccaaggctcgagctcagtacatcaagagcttcgtggagcgcgtgctgaagaacgagcagtacatggtgcacctgactcctgaggagaagtctgccgttactgccctgtggggcaaggtgaacgtggatgaagttggtggtgaggccctgggcaggtaagtcgacgtgggagattctgcctcggacagagagaaactctgctgtgtctgagagttgatctccctatagtgaccctgccttcttgccccgggacgaaatgagagaaatcgtaacgggagtttacgaggcagacaggtactgactctctcttttcccctgcaggctgctggtggtctacccttggacccagaggttctttgagtcctttggggatctgtccactcctgatgctgttatgggcaaccctaaggtgaaggctcatggcaagaaagtgctcggtgcctttagtgatggcctggctcacctggacaacctcaagggcacctttgccacactgagtgagctgcactgtgacaagctgcacgtggatcctgagaacttcagggtgagtctgatgggcacctcctgggtttccttcccctggctattctgctcaaccttcctatcagaaaaaaaggggaagcgattctagggagcagtctccatgactgtgtgtggagtgttgacaagagttcggatattttattctctactcagaattgctgctccccctcactctgttctgtgttgtcatttcctctttctttggtaagcttttaatttccagttgcattttactaaattaattaagctggttatttacttcccatcctgatatcagcttcccctcctcctttcctcccagtccttctctctctcctctctctttctctaatcctttcctttccctcagttcatttcttcttctttgatctacgtttgtttgtctttttaaatattgccttgtaacttgctcagaggacaaggaagatatgtccctgtttcttctcatagctctcaagaatagtagcataattggcttttatgccagggtgacaggggaagaatatattttacatataaattctgtttgacataggattcttataataatttgtcagtagtttaaggttgcaaacaaatgtctttgtaaataagcctgcagtatctggtatttttgctctacagttatgttgatggttcttccatattcccacagctcctgggcaatatgatcgtgattgtgctgggccaccacctgggcaaggatttcacccccgctgcacaggctgccttccagaaggtggtggctggagtggccactgccctggctcacaagtaccactaaaccccctttcctgctcttgcctgtgaacaatggttaattgttcccaagagagcatctgtcagttgttggcaaaatgatagacatttgaaaatctgtcttctgacaaataaaaagcatttatgttcactgcaatgatgttttaaattatttgtctgtgtcatagaagggtttatgctaagttttcaagatacaaagaagtgagggttcaggtctgaccttggggaaataaatgaattacacttcaaatgtgtgggacagcaagcagtaagccacagatcctattgccatgccctaaacactcagagaaaaattcaacaaatggtttcatttacacactacattatgattacattttatgtaaattatttgtttttttctactcttccacataaatgtctttttttcctcttacctacccagcacttcacagttctcaagccaataatttttcttttgtaaaactaccattattctctaaacttttccctctgtgtttaccaagcaacattatttatcttttcataaatcctgttgccttagacagcttcagtagcaatagaggtaggattaaggagagaatagaagtgccctgtttgtcataccatgcctgcacagtcaatagtcactatgggatttcaaatggcactttgcctgggacctttacacttcacaccatactctggcttgagttaggagttaagaatgagagaaatataagtctagagagaataagaatatctagtttttaaggctcattactggggtcttatgaaatttccataataccctgtaaatggaagcatttattttttcaataaatctatcttgaatatccagtgtgggttaggattaaatctctccttcatacagttggactgcttttatttatatggagttactagagttaattcactggccgtcgttttacaacgtcgtgactgggaaaaccctggcgttacccaacttaatcgccttgcagcacatccccctttcgccagctggcgtaatagcgaagaggcccgcaccgatcgcccttcccaacagttgcgcagcctgaatggcgaatggcgcctgatgcggtattttctccttacgcatctgtgcggtatttcacaccgcatatggtgcactctcagtacaatctgctctgatgccgcatagttaagccagccccgacacccgccaacacccgctgacgcgccctgacgggcttgtctgctcccggcatccgcttacagacaagctgtgaccgtctccgggagctgcatgtgtcagaggttttcaccgtcatcaccgaaacgcgcgagacgaaagggcctcgtgatacgcctatttttataggttaatgtcatgataataatggtttcttagacgtcaggtggcacttttcggggaaatgtgcgcggaacccctatttgtttatttttctaaatacattcaaatatgtatccgctcatgagacaataaccctgataaatgcttcaataatattgaaaaaggaagagtatgagtattcaacatttccgtgtcgcccttattcccttttttgcggcattttgccttcctgtttttgctcacccagaaacgctggtgaaagtaaaagatgctgaagatcagttgggtgcacgagtgggttacatcgaactggatctcaacagcggtaagatccttgagagttttcgccccgaagaacgttttccaatgatgagcacttttaaagttctgctatgtggcgcggtattatcccgtattgacgccgggcaagagcaactcggtcgccgcatacactattctcagaatgacttggttgagtactcaccagtcacagaaaagcatcttacggatggcatgacagtaagagaattatgcagtgctgccataaccatgagtgataacactgcggccaacttacttctgacaacgatcggaggaccgaaggagctaaccgcttttttgcacaacatgggggatcatgtaactcgccttgatcgttgggaaccggagctgaatgaagccataccaaacgacgagcgtgacaccacgatgcctgtagcaatggcaacaacgttgcgcaaactattaactggcgaactacttactctagcttcccggcaacaattaatagactggatggaggcggataaagttgcaggaccacttctgcgctcggcccttccggctggctggtttattgctgataaatctggagccggtgagcgtgggtctcgcggtatcattgcagcactggggccagatggtaagccctcccgtatcgtagttatctacacgacggggagtcaggcaactatggatgaacgaaatagacagatcgctgagataggtgcctcactgattaagcattggtaactgtcagaccaagtttactcatatatactttagattgatttaaaacttcatttttaatttaaaaggatctaggtgaagatcctttttgataatctcatgaccaaaatcccttaacgtgagttttcgttccactgagcgtcagaccccgtagaaaagatcaaaggatcttcttgagatcctttttttctgcgcgtaatctgctgcttgcaaacaaaaaaaccaccgctaccagcggtggtttgtttgccggatcaagagctaccaactctttttccgaaggtaactggcttcagcagagcgcagataccaaatactgtccttctagtgtagccgtagttaggccaccacttcaagaactctgtagcaccgcctacatacctcgctctgctaatcctgttaccagtggctgctgccagtggcgataagtcgtgtcttaccgggttggactcaagacgatagttaccggataaggcgcagcggtcgggctgaacggggggttcgtgcacacagcccagcttggagcgaacgacctacaccgaactgagatacctacagcgtgagctatgagaaagcgccacgcttcccgaagggagaaaggcggacaggtatccggtaagcggcagggtcggaacaggagagcgcacgagggagcttccagggggaaacgcctggtatctttatagtcctgtcgggtttcgccacctctgacttgagcgtcgatttttgtgatgctcgtcaggggggcggagcctatggaaaaacgccagcaacgcggcctttttacggttcctggccttttgctggccttttgctcacatgttctttcctgcgttatcccctgattctgtggataaccgtattaccgcctttgagtgagctgataccgctcgccgcagccgaacgaccgagcgcagcgagtcagtgagcgaggaagcggaaga

SEQ ID NO: 23 - DNA, 18 bp, synthetic construct
  misc_feature 1..18: note = "Description of Artificial Sequence: Synthetic oligonucleotide"
  misc_feature 1..18: note = "5SFwd"
  source 1..18: mol_type = other DNA
gccataccaccctgaacg

SEQ ID NO: 24 - DNA, 20 bp, synthetic construct
  misc_feature 1..20: note = "Description of Artificial Sequence: Synthetic oligonucleotide"
  misc_feature 1..20: note = "5SRev"
  source 1..20: mol_type = other DNA
agcttccgagatcagacgag

SEQ ID NO: 25 - DNA, 17 bp, synthetic construct
  misc_feature 1..17: note = "Description of Artificial Sequence: Synthetic oligonucleotide"
  misc_feature 1..17: note = "hGl193-209AS"
  source 1..17: mol_type = other DNA
ccgagcactttcttgcc

SEQ ID NO: 26 - DNA, 20 bp, synthetic construct
  misc_feature 1..20: note = "Description of Artificial Sequence: Synthetic oligonucleotide"
  misc_feature 1..20: note = "U6Rev"
  source 1..20: mol_type = other DNA
aatatggaacgcttcacgaa

SEQ ID NO: 27 - DNA, 51 bp, synthetic construct
  misc_feature 1..51: note = "Description of Artificial Sequence: Synthetic oligonucleotide"
  misc_feature 1..51: note = "pug-NBD1-F1HindIII"
  source 1..51: mol_type = other DNA
attaagcttgtgtgggagattcttcttcggacagagagaaactctgctgtg

SEQ ID NO: 28 - DNA, 60 bp, synthetic construct
  misc_feature 1..60: note = "Description of Artificial Sequence: Synthetic oligonucleotide"
  misc_feature 1..60: note = "pug-NBD1-R1"
  source 1..60: mol_type = other DNA
ctgctgtgtctgaaagaagatctccctatagtgaccctgccttaccttctccgggacgaa

SEQ ID NO: 29 - DNA, 58 bp, synthetic construct
  misc_feature 1..58: note = "Description of Artificial Sequence: Synthetic oligonucleotide"
  misc_feature 1..58: note = "pug-NBD1-R2BamHI"
  source 1..58: mol_type = other DNA
atggatccacctgtctgcctcgtattcttccgttacgatttctctcatttcgtcccgg

SEQ ID NO: 30 - DNA, 51 bp, synthetic construct
  misc_feature 1..51: note = "Description of Artificial Sequence: Synthetic oligonucleotide"
  misc_feature 1..51: note = "pug-mmidua-F1HindIII"
  source 1..51: mol_type = other DNA
attaagcttgtgtgggagattctgcctcggacagagagaaactctgctgtg

SEQ ID NO: 31 - DNA, 60 bp, synthetic construct
  misc_feature 1..60: note = "Description of Artificial Sequence: Synthetic oligonucleotide"
  misc_feature 1..60: note = "pug-mmidua-R1"
  source 1..60: mol_type = other DNA
ttcgtcccggggcagagaaggcagggtcactatagggagatcaactctcagacacagcag

SEQ ID NO: 32 - DNA, 58 bp, synthetic construct
  misc_feature 1..58: note = "Description of Artificial Sequence: Synthetic oligonucleotide"
  misc_feature 1..58: note = "pug-mmidua-R2BamHI"
  source 1..58: mol_type = other DNA
atggatccacctgtctgcctcgtaaactcccgttacgatttctctcatttcgtcccgg

SEQ ID NO: 33 - DNA, 58 bp, synthetic construct
  misc_feature 1..58: note = "Description of Artificial Sequence: Synthetic oligonucleotide"
  misc_feature 1..58: note = "SDM-GL39-SWAPto-NBD1-1"
  source 1..58: mol_type = other DNA
tggtggacaatatagttctttgagaaggtggaatcacatttggggatctgtccactcc

SEQ ID NO: 34 - DNA, 58 bp, synthetic construct
  misc_feature 1..58: note = "Description of Artificial Sequence: Synthetic oligonucleotide"
  misc_feature 1..58: note = "SDM-GL39-SWAPto-NBD1-2"
  source 1..58: mol_type = other DNA
ccaaatgtgattccaccttctcaaagaactatattgtccaccagcagcctaagggtgg

SEQ ID NO: 35 - DNA, 16 bp, synthetic construct
  misc_feature 1..16: note = "Description of Artificial Sequence: Synthetic oligonucleotide"
  misc_feature 1..16: note = "NBD1PSU-202Fwd"
  source 1..16: mol_type = other DNA
ctggagccttcagagg

SEQ ID NO: 36 - DNA, 19 bp, synthetic construct
  misc_feature 1..19: note = "Description of Artificial Sequence: Synthetic oligonucleotide"
  misc_feature 1..19: note = "NBD1PSU+40(491-509)Rev"
  source 1..19: mol_type = other DNA
gctcttgctaaagaaattc

SEQ ID NO: 37 - protein, 31 aa, synthetic construct
  REGION 1..31: note = "Description of Artificial Sequence: Synthetic polypeptide"
MVHLTPEEKSAVTALWGKVNVDEVGGEALGR

SEQ ID NO: 38 - protein, 74 aa, synthetic construct
  REGION 1..74: note = "Description of Artificial Sequence: Synthetic polypeptide"
LLVVYPWTQRFFESFGDLSTPDAVMGNPKVKAHGKKVLGAFSDGLAHLDNLKGTFATLSELHCDKLHVDPENFR

SEQ ID NO: 39 - protein, 31 aa, synthetic construct; identical to SEQ ID NO: 37
  REGION 1..31: note = "Description of Artificial Sequence: Synthetic polypeptide"

SEQ ID NO: 40 - protein, 74 aa, synthetic construct; identical to SEQ ID NO: 38
  REGION 1..74: note = "Description of Artificial Sequence: Synthetic polypeptide"

SEQ ID NO: 41 - protein, 105 aa, synthetic construct
MVHLTPEEKSAVTALWGKVNVDEVGGEALGRLLVVYPWTQRFFESFGDLSTPDAVMGNPKVKAHGKKVLGAFSDGLAHLDNLKGTFATLSELHCDKLHVDPENFR

SEQ ID NO: 42 - protein, 105 aa, synthetic construct; identical to SEQ ID NO: 41